European Patent Specification EP 3 874 055 B1, published June 14, 2023. Title: Enzymatic method for preparation of UDP-galactose. Applicant: Max-Planck-Gesellschaft zur Foerderung der Wissenschaften e.V. The sequence listing filed with the application follows.

SEQUENCE LISTING (9 sequences)

SEQ ID NO: 1 - protein, 416 aa, Bifidobacterium infantis ATCC 15697
  galactokinase
MTAVEFIEPLTHEEGVSQATKLFVDTYGAAPEGVWAAPGRVNLIGEHTDYNAGLCLPIALPHRTFIALKPREDTKVRVVSGVAPDKVAEADLDGLKARGVDGWSAYPTGVAWALRQAGFDKVKGFDAAFVSCVPLGSGLSSSAAMTCSTALALDDVYGLGYGDSDAGRVTLINAAIKSENEMAGASTGGLDQNASMRCTEGHALLLDCRPELTPLENVSQQEFDLDKYNLELLVVDTQAPHQLNDGQYAQRRATCEEAAKILGVANLRVTADGISKADDQFQALKETLDALPDETMKKRVRHVVTEIERVRSFVRAFAQGDIKAAGRLFNASHDSLAADYEVTVPELDIAVDVARKNGAYGARMTGGGFGGSIIALVDKGQGHEIAQKIADRFEKEGFNAPRALPAFAAASASREA

SEQ ID NO: 2 - protein, 202 aa, Arabidopsis thaliana [sequence omitted]

SEQ ID NO: 3 - protein, 301 aa, Ruegeria pomeroyi
  polyphosphate kinase 3
MNRNGSTKDPRRMTGAATGEISRYFNDKAPKDIRRAIEKADKDDILSTTYPYDAEMTAKDYRAQMEALQIELVKLQAWIKQSGARVALLFEGRDAAGKGGTIKRFRENLNPRGARVVALSKPTEAERSQWYFQRYIQHLPSAGELVFYDRSWYNRGVVEHVFGWCDEEQRERFFRQVMPFEHDLVDDGIHLFKFWLNVGRAEQLRRFHDRERDPLKQWKLSPVDIAGLDKWEAYTTAISQTLTRSHSDRAPWTVIRSDDKKRARLAAIRTVLSGIDYDNKDRAAVGQPDAAICGGPDIWDA

SEQ ID NO: 4 - protein, 302 aa, E. coli K-12 MG1655
  glucose 1-phosphate uridylyltransferase
MAAINTKVKKAVIPVAGLGTRMLPATKAIPKEMLPLVDKPLIQYVVNECIAAGITEIVLVTHSSKNSIENHFDTSFELEAMLEKRVKRQLLDEVQSICPPHVTIMQVRQGLAKGLGHAVLCAHPVVGDEPVAVILPDVILDEYESDLSQDNLAEMIRRFDETGHSQIMVEPVADVTAYGVVDCKGVELAPGESVPMVGVVEKPKADVAPSNLAIVGRYVLSADIWPLLAKTPPGAGDEIQLTDAIDMLIEKETVEAYHMKGKSHDCGNKLGYMQAFVEYGIRHNTLGTEFKAWLEEEMGIKK

SEQ ID NO: 5 - protein, 175 aa, Pasteurella multocida subsp. multocida str. Pm70
  inorganic diphosphatase
MGLETVPAGKALPDDIYVVIEIPANSDPIKYEVDKESGALFVDRFMATAMFYPANYGYVNNTLSLDGDPVDVLVPTPYPLQPGSVIRCRPVGVLKMTDEAGSDAKVVAVPHSKLTKEYDHIKDVNDLPALLKAQIQHFFESYKALEAGKWVKVDGWEGVDAARQEILDSFERAKK

SEQ ID NO: 6 - protein, 304 aa, Pseudomonas aeruginosa
  1-domain polyphosphate kinase 2
MDSYGDTSGRIGRDWLDRHDEELEQELLDDELNLDELFGPEQEDAPGELSRRRYFRELFRLQRELVKLQNWVVHTGHKVVILFEGRDAAGKGGVIKRITQRLNPRVCRVAALPAPNDREQTQWYFQRYVSHLPAGGEIVLFDRSWYNRAGVERVMGFCNDEQYEEFFRSVPEFEKMLARSGIQLLKYWFSISDAEQHLRFLSRIHDPLKQWKLSPMDLESRRRWEAYTKAKETMLERTHIPEAPWWVVQADDKKRARLNCIHHLLQQMPYREVPQPPVHLPERLRHADYVRHPTPGEIIVPEVY

SEQ ID NO: 7 - protein, 496 aa, Pseudomonas aeruginosa
  2-domain polyphosphate kinase 2
MFESAEVGHSIDKDTYEKAVIELREALLEAQFELKQQARFPVIILINGIEGAGKGETVKLLNEWMDPRLIEVQSFLRPSDEELERPPQWRFWRRLPPKGRTGIFFGNWYSQMLYARVEGHIKEAKLDQAIDAAERFERMLCDEGALLFKFWFHLSKKQLKERLKALEKDPQHSWKLSPLDWKQSEVYDRFVHYGERVLRRTSRDYAPWYVVEGADERYRALTVGRILLEGLQAALATKERAKRQPHAAPLVSSLDNRGLLDSLDLGQYLDKDAYKEQLAAEQARLAGLIRDKRFRQHSLVAVFEGNDAAGKGGAIRRVTDALDPRQYHIVPIAAPTEEERAQPYLWRFWRHIPARRQFTIFDRSWYGRVLVERIEGFCAPADWLRAYGEINDFEEQLSEYGIIVVKFWLAIDKQTQMERFKEREKTPYKRYKITEEDWRNRDKWDQYVDAVGDMVDRTSTEIAPWTLVEANDKRFARVKVLRTINDAIEAAYKKDK

SEQ ID NO: 8 - protein, 416 aa, Bifidobacterium longum
  galactokinase
MTAVEFIEPLTHEEGVSQATKLFVDTYGAAPEGVWAAPGRVNLIGEHTDYNAGLCLPIALPHRTFIALKPREDTKVRVVSDVAPDKVAEADLDGLKARGVDGWSAYPTGVAWALRQAGFDKVKGFDAAFVSCVPLGSGLSSSAAMTCSTALALDDVYGLGYGDSDAGRVTLINAAIKSENEMAGASTGGLDQNASMRCTAGHALLLDCRPELTPLENVSQQEFDLDKYNLELLVVDTQAPHQLNDGQYAQRRATCEEAAKILGVANLRVTADGISKADDQFQALKETLDALPDETMKKRVRHVVTEIERVRSFVRAFAQGDIKAAGRLFNASHDSLAADYEVTVPELDIAVDVARKNGAYGARMTGGGFGGSIIALVDKGRSQEVAQKIADEFEKQGFHAPRALAAYAAPSASREA

SEQ ID NO: 9 - protein, 213 aa, Escherichia coli K-12
  uridine/cytidine kinase
MTDQSHQCVIIGIAGASASGKSLIASTLYRELREQVGDEHIGVIPEDCYYKDQSHLSMEERVKTNYDHPSAMDHSLLLEHLQALKRGSAIDLPVYSYVEHTRMKETVTVEPKKVIILEGILLLTDARLRDELNFSIFVDTPLDICLMRRIKRDVNERGRSMDSVMAQYQKTVRPMFLQFIEPSKQYADIIVPRGGKNRIAIDILKAKISQFFE